European Patent Application EP 4 382 597 A1, published June 12, 2024. Title: Reagent for beta glucan assay, production method and use thereof. Applicant: 生化学工業株式会社. Application WO. The sequence listing filed with the application follows.

SEQUENCE LISTING (72 sequences)

SEQ ID NO: 1 - protein, 394 aa, Tachypleus tridentatus
MKVLLLVAFLLGTTLAYPQDDDGPVWGGSSNDNDDGGISSRVGNPQSGFGNCECVPYYLCKDNNIIIDGSGLLDPRKKPVASKEPKLSARLGPEGPSGCGPFHVCCIAPETSTVKPYTHQCGFRNVNGINKRILSPNGKDLSEFGEWPWQGAVLKVEGKVNIFQCGAVLIDSYHLLTVAHCVYKFTLENAFPLKVRLGEWDTQNTNEFLKHEDYEVEKIYIHPKYDDERKNLWDDIAILKLKAEVSFGPHIDTICLPNNQEHFAGVQCVVTGWGKNAYKNGSYSNVLREVHVPVITNDRCQELLRKTRLSEWYVLYENFICAGGESNADSCKGDGGGPLTCWRKDGTYGLAGLVSWGINCGSPNVPGVYVRVSNYLDWITKITGRPISDYWPRS

SEQ ID NO: 2 - protein, 376 aa, Tachypleus tridentatus
QDDDGPVWGGSSNDNDDGGISSRVGNPQSGFGNCECVPYYLCKDNNIIIDGSGLLDPRKKPVASKEPKLSARLGPEGPSGCGPFHVCCIAPETSTVKPYTHQCGFRNVNGINKRILSPNGKDLSEFGEWPWQGAVLKVEGKVNIFQCGAVLIDSYHLLTVAHCVYKFTLENAFPLKVRLGEWDTQNTNEFLKHEDYEVEKIYIHPKYDDERKNLWDDIAILKLKAEVSFGPHIDTICLPNNQEHFAGVQCVVTGWGKNAYKNGSYSNVLREVHVPVITNDRCQELLRKTRLSEWYVLYENFICAGGESNADSCKGDGGGPLTCWRKDGTYGLAGLVSWGINCGSPNVPGVYVRVSNYLDWITKITGRPISDYWPRS

SEQ ID NO: 3 - protein, 394 aa, Tachypleus tridentatus
MKVLLLVAFLLGTTLAYPQDDDGPVWGGSSNDNDDGGISSRVGNPQSGFGNCECVPYYLCKDNNIIIDGSGLLDPRKKPVASKEPKLSARLGPEGPSGCGPFHVCCIAPETSTVKPYTHQCGFRNVNGINKRILSPNGKDLSEFGEWPWQGAVLKVEGKVNIFQCGAVLIDSYHLLTVAHCVYKFTLENAFPLKVRLGEWDTQNTNEFLKHEDYEVEKIYIHPKYDDERKNLWDDIAILKLKAEVSFGPHIDTICLPNNQEHFAGVQCVVTGWGKNAYKNGSYSNVLREVHVPVITNDRCQELLRKTRLSEWYVLYENFICAGGESNADSCKGDGGGPLTCWRKDGTYGLAGLVSWGINCGSPNVPGVYVRVANYLDWITKITGRPISDYWPRS

SEQ ID NO: 4 - protein, 376 aa, Tachypleus tridentatus
QDDDGPVWGGSSNDNDDGGISSRVGNPQSGFGNCECVPYYLCKDNNIIIDGSGLLDPRKKPVASKEPKLSARLGPEGPSGCGPFHVCCIAPETSTVKPYTHQCGFRNVNGINKRILSPNGKDLSEFGEWPWQGAVLKVEGKVNIFQCGAVLIDSYHLLTVAHCVYKFTLENAFPLKVRLGEWDTQNTNEFLKHEDYEVEKIYIHPKYDDERKNLWDDIAILKLKAEVSFGPHIDTICLPNNQEHFAGVQCVVTGWGKNAYKNGSYSNVLREVHVPVITNDRCQELLRKTRLSEWYVLYENFICAGGESNADSCKGDGGGPLTCWRKDGTYGLAGLVSWGINCGSPNVPGVYVRVANYLDWITKITGRPISDYWPRS

SEQ ID NO: 5 - protein, 413 aa, Tachypleus tridentatus
MGILPSPGMPALLSLVSLLSVLLMGCVAETGQDDDGPVWGGSSNDNDDGGISSRVGNPQSGFGNCECVPYYLCKDNNIIIDGSGLLDPRKKPVASKEPKLSARLGPEGPSGCGPFHVCCIAPETSTVKPYTHQCGFRNVNGINKRILSPNGKDLSEFGEWPWQGAVLKVEGKVNIFQCGAVLIDSYHLLTVAHCVYKFTLENAFPLKVRLGEWDTQNTNEFLKHEDYEVEKIYIHPKYDDERKNLWDDIAILKLKAEVSFGPHIDTICLPNNQEHFAGVQCVVTGWGKNAYKNGSYSNVLREVHVPVITNDRCQELLRKTRLSEWYVLYENFICAGGESNADSCKGDGGGPLTCWRKDGTYGLAGLVSWGINCGSPNVPGVYVRVANYLDWITKITGRPISDYWPRSHHHHHH

SEQ ID NO: 6 - protein, 385 aa, Tachypleus tridentatus
ETGQDDDGPVWGGSSNDNDDGGISSRVGNPQSGFGNCECVPYYLCKDNNIIIDGSGLLDPRKKPVASKEPKLSARLGPEGPSGCGPFHVCCIAPETSTVKPYTHQCGFRNVNGINKRILSPNGKDLSEFGEWPWQGAVLKVEGKVNIFQCGAVLIDSYHLLTVAHCVYKFTLENAFPLKVRLGEWDTQNTNEFLKHEDYEVEKIYIHPKYDDERKNLWDDIAILKLKAEVSFGPHIDTICLPNNQEHFAGVQCVVTGWGKNAYKNGSYSNVLREVHVPVITNDRCQELLRKTRLSEWYVLYENFICAGGESNADSCKGDGGGPLTCWRKDGTYGLAGLVSWGINCGSPNVPGVYVRVANYLDWITKITGRPISDYWPRSHHHHHH

SEQ ID NO: 7 - protein, 394 aa, Limulus polyphemus
MKVLLLMTFLFETALAYPQDDDGPIWGGSNSDNDDGSINSRVDNPHSGFGNCECVPYYVCKDDNIITDGSGVLDPRKKPVPSKEPDLFAHLSPEGRRGCGNFHVCCIAPTTSTVKPYTRQCGFRKVNGINKRILSPNGKNLSEFGEWPWQGAVLKVEGKVNIFQCGAVLIDSFHLLTVAHCVYRFTLENAFPLKVRLGEWDTQNTNEFLKHEDYEVEKISIHSKYNHERKNLWDDIAILKLKVEVSFGPHIDTICLPKYQEKFEGVQCVVTGWGKNAYKNGSYTNVLRKAHVPVISNDKCQQLLRKTRLSKWFILYENFICAGGESNADSCKGDGGGPLACWRKDGTYGLAGLVSWGIGCGSPNVPGVYVRVTNYLDWITEVTGRPISEYWPRS

SEQ ID NO: 8 - protein, 376 aa, Limulus polyphemus
QDDDGPIWGGSNSDNDDGSINSRVDNPHSGFGNCECVPYYVCKDDNIITDGSGVLDPRKKPVPSKEPDLFAHLSPEGRRGCGNFHVCCIAPTTSTVKPYTRQCGFRKVNGINKRILSPNGKNLSEFGEWPWQGAVLKVEGKVNIFQCGAVLIDSFHLLTVAHCVYRFTLENAFPLKVRLGEWDTQNTNEFLKHEDYEVEKISIHSKYNHERKNLWDDIAILKLKVEVSFGPHIDTICLPKYQEKFEGVQCVVTGWGKNAYKNGSYTNVLRKAHVPVISNDKCQQLLRKTRLSKWFILYENFICAGGESNADSCKGDGGGPLACWRKDGTYGLAGLVSWGIGCGSPNVPGVYVRVTNYLDWITEVTGRPISEYWPRS

SEQ ID NO: 9 - protein, 396 aa, Limulus polyphemus
MKVLLLMTFLFGTALAYPQDDDGPVWGGSNNDDDDDDGGISSRVGNPQSSFGNCECVPYYLCKDNNIITDGSGVLDPRKKPVPSKEPGLSARLGPEGPSGCGPFHVCCTAPTTSTVKPYTHQCGFRNVNGINKRILSPNGKDLSEFGEWPWQGAVLKVEGKVNIFQCGAVLIDSFHLLTVAHCVYRFTLANAFPLKVRLGEWDTQNTDEFLKHEDYEVEKIYIHSKYNHERKNLWDDIAILKLKVEVSFGPHIDTICLPNYQENFEGVQCVVTGWGKNAYKNGTYSNVLREVHVPVISNDKCEQLLKETRLSKWFVLYENFTCAGGESNADSCKGDGGGPLACWRKDGTYALAGLVSWGIDCGSPNVPGVYVRVAKYLDWIAQITGRPVTDYWPRS

SEQ ID NO: 10 - protein, 378 aa, Limulus polyphemus
QDDDGPVWGGSNNDDDDDDGGISSRVGNPQSSFGNCECVPYYLCKDNNIITDGSGVLDPRKKPVPSKEPGLSARLGPEGPSGCGPFHVCCTAPTTSTVKPYTHQCGFRNVNGINKRILSPNGKDLSEFGEWPWQGAVLKVEGKVNIFQCGAVLIDSFHLLTVAHCVYRFTLANAFPLKVRLGEWDTQNTDEFLKHEDYEVEKIYIHSKYNHERKNLWDDIAILKLKVEVSFGPHIDTICLPNYQENFEGVQCVVTGWGKNAYKNGTYSNVLREVHVPVISNDKCEQLLKETRLSKWFVLYENFTCAGGESNADSCKGDGGGPLACWRKDGTYALAGLVSWGIDCGSPNVPGVYVRVAKYLDWIAQITGRPVTDYWPRS

SEQ ID NO: 11 - protein, 415 aa, Limulus polyphemus
MGILPSPGMPALLSLVSLLSVLLMGCVAETGQDDDGPVWGGSNNDDDDDDGGISSRVGNPQSSFGNCECVPYYLCKDNNIITDGSGVLDPRKKPVPSKEPGLSARLGPEGPSGCGPFHVCCTAPTTSTVKPYTHQCGFRNVNGINKRILSPNGKDLSEFGEWPWQGAVLKVEGKVNIFQCGAVLIDSFHLLTVAHCVYRFTLANAFPLKVRLGEWDTQNTDEFLKHEDYEVEKIYIHSKYNHERKNLWDDIAILKLKVEVSFGPHIDTICLPNYQENFEGVQCVVTGWGKNAYKNGTYSNVLREVHVPVISNDKCEQLLKETRLSKWFVLYENFTCAGGESNADSCKGDGGGPLACWRKDGTYALAGLVSWGIDCGSPNVPGVYVRVAKYLDWIAQITGRPVTDYWPRSHHHHHH

SEQ ID NO: 12 - protein, 387 aa, Limulus polyphemus
ETGQDDDGPVWGGSNNDDDDDDGGISSRVGNPQSSFGNCECVPYYLCKDNNIITDGSGVLDPRKKPVPSKEPGLSARLGPEGPSGCGPFHVCCTAPTTSTVKPYTHQCGFRNVNGINKRILSPNGKDLSEFGEWPWQGAVLKVEGKVNIFQCGAVLIDSFHLLTVAHCVYRFTLANAFPLKVRLGEWDTQNTDEFLKHEDYEVEKIYIHSKYNHERKNLWDDIAILKLKVEVSFGPHIDTICLPNYQENFEGVQCVVTGWGKNAYKNGTYSNVLREVHVPVISNDKCEQLLKETRLSKWFVLYENFTCAGGESNADSCKGDGGGPLACWRKDGTYALAGLVSWGIDCGSPNVPGVYVRVAKYLDWIAQITGRPVTDYWPRSHHHHHH

SEQ ID NO: 13 - protein, 673 aa, Tachypleus tridentatus
MLVLLCCVVLHVGVARICCSHEPKWQLVWSDEFTNGISSDWEFEMGNGLNGWGNNELQYYRRENAQVEGGKLVITAKREDYDGFKYTSARLKTQFDKSWKYGKIEAKMAIPSFRGVWVMFWMSGDNTNYVRWPSSGEIDFIEHRNTNNEKVRGTIHWSTPDGAHAHHNRESNTNGIDYHIYSVEWNSSIVKWFVNGNQYFEVKIQGGVNGKSAFRNKVFVILNMAIGGNWPGFDVADEAFPAKMYIDYVRVYQDASTSSPVGDTSLDGYYFVQNRHSELYLDVTDASNEDGAFLQQWSYSGNENQQFDFEHLENNVYKITNKKSGKSLDVYNFGTENGVRIQQWSYGGARNQQFTVQSVGDGYYKIIPRGSGKLVEVADFSKDAGGKIQQWSDNNQLSGQWKLIKSKSYSKLIQAESYFDSSKVQLEDTSDVGGGKNVKCDNEGAWMAYKDIDFPSSGNYRIEYRVASERAGGKLSLDLNAGSIVLGMLDVPSTGGWQKWTTISHTVNVDSGTYNLGIYVQRASWNINWIKITKIPEQSNLNQGRRNSKLIQAESYFSYSEVQLEDTLDVGGGKNVKCDKEGAWMAYKDIDFPSSGSYRVEYRVASERAGGKLSLDLNAGSIVLGMLDIPSTGGLQKWTTISHIVNVDLGTYNLGIYVQKASWNINWIRITKV

SEQ ID NO: 14 - protein, 309 aa, Tachypleus tridentatus
MDISFLVFITLSMALFSSNVTGTSVTSRVRRGINEKHCGFRPVITRIIGGGIATPHSWPWMVGIFKVNPHRFLCGGSIINKVSVVTAAHCLVTQFGNRQNYSIFVRVGAHDIDNSGTNYQVDKVIVHQGYKHHSHYYDIGLILLSKPVEYNDKIQPVCIPEFNKPHVNLNNIKVVITGWGVTGKATEKRNVLRELELPVVTNEQCNKSYQTLPFSKLNRGITNDMICAGFPEGGKDACQGDSGGPLMYQNPTTGRVKIVGVVSFGFECARPNFPGVYTRLSSYVNWLQEITFGQSLASLFEVVPIFIPE

SEQ ID NO: 15 - protein, 668 aa, Limulus polyphemus
MLVLLCCVVLHVGVARICCSQEPKWKLVWSDEFTNGISSDWEFETGNGPNGWGNNELQYYRRENTRVEGGKLIITAKEEDYEGFRYTSAKLKTQFNKPWKDGKIEARMSIPSFRGVWVAFWMLGDITDTDSWPSSGEIDFEEHINTNNEVRGTIHWSTSDDADTLHGRGTNTDYHIYSVEWNSSVIRWFVDGNQYFDVNIQRGATGTNAFHNNVFVILNMAIGGNWPGFNVADEAFPANMYVDYVRVYQDANTPSPVDVTHLSGYYFLQNRHSELYLDVSGSSNEDGAFLQQWPYSGNANQQFDFVHLGNKVYKIINKNSGKSLDVYELGTDNGVRIQQWSYGGGYNQQFIVQDVGDGYYKIFARSTGKLVEVADLNKDPGGKIQQWSDDGQLSGQWKLIRNKANSKLIQAESYFASSKVQLEDTSDVGGGKNVKCDNEGAWMAYKDINFPSSGTYQVEYRVASERAGGMLSLDLNAGSIVLGMLNVPSTGGLQKWTTISHTVNVSSGTYNLGISVQRPGWNINWINITKVSSQLKSIPSTNSRVIQAESYFDSSKVQLEDTSDVGGGKNVKCDTKGAWMAYKDINFPSSGSYQIEYRVASERAGGKLSLDLNAGSIVLGMLDVPSTGGWQKWTTISHTVKVDSGTYNLGIYVQQPGWNINWIKITKV

SEQ ID NO: 16 - protein, 666 aa, Limulus polyphemus
MFLCYVVLYVGVAGIYCSQEPKWKLVWSDEFTNGISSDWEFETGNGPNGWGNNELQYYRRENTRVEGGKLIITAKEEDYEGFRYTSAKLKTQFNKPWKDGKIEARMSIPSFRGVWVAFWMLGDITDTDSWPSSGEIDFEEHINTNNEVRGTIHWSTSDDADTLHGRGTNTDYHIYSVEWNSSVIRWFVDGNQYFEVNIQRGATGTNAFHNNVFVILNMAIGGNWPGFNVADEAFPANMYVDYVRVYQDANTPSPVDVTHLSGYYFLQNRHSELYLDVSGSSNEDGAFLQQWPYSGNANQQFDFVHLGNKVYKIINKNSGKSLDVYELGTDNGVRIQQWSYGGGYNQQFIVQDVGDGYYKIFARSTGKLVEVADLNKDPGGKIQQWSDDGQLSGQWKLIRNKANSKLIQAESYFASSKVQLEDTSDVGGGKNVKCDNEGAWMAYKDINFPSSGTYQVEYRVASERAGGMLSLDLNAGSIVLGMLNVPSTGGLQKWTTISHTVNVSSGTYNLGISVQRPGWNINWINITKVSSQLKSIPSTNSRVIQAESYFDSSKVQLEDTSDVGGGKNVKCDTKGAWMAYKDINFPSSGSYQIEYRVASERAGGKLSLDLNAGSIVLGMLDVPSTGGWQKWTTISHTVKVDSGTYNLGIYVQQPGWNINWIKITKV

SEQ ID NO: 17 - protein, 670 aa, Limulus polyphemus
MFLCYVVLVVGVTGICCSQETNWKLVWSDEFTNGISSDWEFETGNGPNGWGNNELQYYRRENARVEGGKLIITAKKEDYEGFRYTSAKLKTQFNKPWKDGKIEARMSIPSFRGVWVAFWMLGDITDTDSWPSSGEIDFKEHINTNNEVRGTIHWSTSDGAHTHHGRGTNTDYHIYSVEWNSSVIRWFVDGNQYFEVNIQRGATGTNAFHNKVFVILNMAIGGNWPGFNVADEAFPANMYVDYVRVYQDANTPSPVDVDVTDLSGYYFLQNRHSELYLDVSFSSNKDGAFLQQWPYNGNANQQFDFVHLGNNIYKITNKNSGKSLDVYNVGTENGVRIQQMPYRGSYNQQFIVQDVGDGYYKIFARNSRKLVEVADFNKDPGGKIQQWSDDGQISGQWKLIRNKVNSKVIQAESYFASLGVQLEDTSDVGGGKNVKCDTEGAWMAYKDINFPSSGSYQVEYRVASERAGGKLSLDLNAGSIVLGMLNVPSTGGWQKWTTISHTVKVDSGTYNLGIYVQRPRWNINWIKITEAPGQSKPIQRSDTDSKVIQAESYFASSKVQLEDTSDVGGGKNVKCDNEGAWMAYKDINFPSSGSYQIEYRVASERAGGKLSLDLNAGSIVLGMLDVPSTGGWQKWTTISHTVNVSSGTYNLGIYVQRAAWNINWIKITKV

SEQ ID NO: 18 - protein, 308 aa, Limulus polyphemus
MKTTLWTFFALAMALFSINVTASEMSVTSRVRREINEEHCGIRPTAPRIIKGRISIPHSWPWMVGIFQVDPLLFICGGTIINKVSVVTAAHCLVTQSGNRQNSSIVVRVGAHDIDNSGIDYHVDKIIVHQDYKYRSQYYDIGLILLSKRIEYNYKVRPVCIPELNKLNVNLNNKEVVVIGWGVTERGSEKHNVLRELELPVVTNELCNKSYQTISFSGLNRGITDDMICAGYQEGGRDSCEGDSGGPLMYHDPTTGRVELVGVVSFGFGCARPNFPGVYTRLSSYGNWFQKVTFGYLLATLFEVVPVF

SEQ ID NO: 19 - protein, 308 aa, Limulus polyphemus
MKTTLWTFFALAMALFSINVTASEMSVTSRVRREINEEHCGIRPTAPRIIKGRISIPHSWPWMVGIFQVDPLLFICGGTIINKVSVVTAAHCLVTQSGNRQNSSIVVRVGAHDIDNSGIDYHVDKIIVHQDYKYRSQYYDIGLILLSKPIEYNYKVRPVCIPELNKLNVNLNNKEVVVIGWGVTERGSEKYNVLRELELPVVTNELCNKSYQTISFSGLNRGITDDMICAGYQEGGRDSCEGDSGGPLMYHDPTTGRVELVGVVSFGFGCARPNFPGVYTRLSSYGNWFQKVTFGYLLATLFEVVPVF

SEQ ID NO: 20 - protein, 308 aa, Limulus polyphemus
MKTTLWTFFALAMALFSINVTASEMSVTSRVRREINEEHCGIRPTAPRIIKGRISIPHSWPWMVGIFQVDPLLFICGGTIINKVSVVTAAHCLVTQSGNRQNYSIVVRVGAHDIDNSGIDYHVDKIIVHQDYKYRSQYYDIGLILLSKPIEYNYKVRPVCIPELNKLNVNLNNKEVVVIGWGVTERGSEKHNVLRELELPVVTNELCNKSYQTISFSGLNRGITDDMICAGYQEGGRDSCEGDSGGPLMYHDPTTGGVELVGVVSFGFGCARPNFPGVYTRLSSYGNWFQKVTFGYLLATLFEVVPVF

SEQ ID NO: 21 - protein, 308 aa, Limulus polyphemus
MKTTLWTFFALAMALFSINVTASEMSVTSRVRREINEEHCGIRPTAPRIIKGRISIPHSWPWMVGIFQVDPLLFICGGTIINKVSVVTAAHCLVTQSGNRQNYSIVVRVGAHDIDNSGIDYHVDKIIVHQDYKYRSQYYDIGLILLSKPIEYNYKVRPVCIPELNKLNVNLNNKEVVVIGWGVTERGSEKYNVLRELELPVVTNELCNKSYQTISFSGLNRGITDDMICAGYQEGGRDSCEGDSGGPLMYHDPTTGRVELVGVVSFGFGCARPNFPGVYTRLSSYGNWFQKVTFGYLLATLFEVVPVF

SEQ ID NO: 22 - protein, 308 aa, Limulus polyphemus
MKTTLWTFFALAMALFSINVTASEMSVTSRVRREINEEHCGIRPTAPRIIKGRISIPHSWPWMVGIFQVDPLLFICGGTIINKVSVVTAAHCLVTQSGNRQNSSIVVRVGAHDIDNSGIDYHVDKIIVHQDYKYRSQYYDIGLILLSKRIEYNYKVRPVCIPELNKLNVNLNNKEVVVIGWGVTERGSEKYNVLRELELPVVTNELCNKSYQTISFSGLNRGITDDMICAGYQEGGRDSCEGDSGGPLMYHDPTTGRVELVGVVSFGFGCARPNFPGVYTRLSSYGNWFQKVTFGYLLATLFEVVPVF

SEQ ID NO: 23 - protein, 308 aa, Limulus polyphemus
MKTTLWTFFALAMALFSINVTASEMSVTSRVRREINEEHCGIRPTAPRIIKGRISIPHSWPWMVGIFQVDPLLFICGGTIINKVSVVTAAHCLVTQSGNRQNYSIVVRVGAHDIDNSGIDYHVDKIIVHQDYKYRSQYYDIGLILLSKPIEYNYKVRPVCIPELNKLNVNLNNKEVVVIGWGVTERGSEKHNVLRELELPVVTNELCNKSYQTISFSGLNRGITDDMICAGYQEGGRDSCEGDSGGPLMYHDPTTGRVELVGVVSFGFGCARPNFPGVYTRLSSYGNWFQKVTFGYLLATLFEVVPVF

SEQ ID NO: 24 - protein, 375 aa, Tachypleus tridentatus
MLVNNVFSLLCFPLLMSVVRCSTLSRQRRQFVFPDEEELCSNRFTEEGTCKNVLDCRILLQKNDYNLLKESICGFEGITPKVCCPKSSHVISSTQAPPETTTTERPPKQIPPNLPEVCGIHNTTTTRIIGGREAPIGAWPWMTAVYIKQGGIRSVQCGGALVTNRHVITASHCVVNSAGTDVMPADVFSVRLGEHNLYSTDDDSNPIDFAVTSVKHHEHFVLATYLNDIAILTLNDTVTFTDRIRPICLPYRKLRYDDLAMRKPFITGWGTTAFNGPSSAVLREVQLPIWEHEACRQAYEKDLNITNVYMCAGFADGGKDACQGDSGGPMMLPVKTGEFYLIGIVSFGKKCALPGFPGVYTKVTEFLDWIAEHMV

SEQ ID NO: 25 - protein, 375 aa, Limulus polyphemus
MLVNNMFSLLCFPLLMSMFSCSSLGRQRRQFVFPDDEESCSNRFTNDGICKDVLNCRDLLQKNDYNLLKESICGFEGITPKVCCPKQSIVNPITEAPPKTTTTERPPIRIPSNLPKQCGNRNITTTRIIGGQEATPGAWPWMAAVYIKQGGIRSVQCGGALVTNRHVITASHCVVNSLGTDVMRADVFSVRLGEHNLYSTNDSSDPIDFAVTSVKHHENFVLATYLNDIAILKLNDTVTFTHKIKPICLPYESLRYEDLAMRNPFVAGWGTTAFNGPSSAVLREVQLPIWGHEPCRQAYEKDLNITNVYMCAGYADGGKDACQGDSGGPMMLPDKSGNFYLVGIVSFGKKCALPGFPGVYTKVTEFLDWIAVNMV

SEQ ID NO: 26 - DNA, 1185 bp, Tachypleus tridentatus
  source 1..1185: mol_type = genomic DNA
atgaaagtgttgttgttggtggctttccttttgggaacgacgttggcttatccacaagacgatgacgggccagtctggggtggttcaagcaacgataatgatgatggtggtattagcagtcgcgttggcaacccccaatctggttttggtaactgtgagtgtgtaccttattacttgtgtaaggataataatattatcattgatggttctggcttactcgaccctagaaaaaaaccagtagcctccaaagaacctaaattgtctgcacgcctaggtccagaaggtccaagtgggtgtggtccttttcacgtatgctgtattgcaccagaaacatccacagtaaaaccatatactcatcaatgtggcttcagaaacgtcaatggaatcaacaagcgtattttgagtcctaatggtaaagatctatctgagtttggagagtggccttggcagggagctgtattgaaagtcgaaggcaaagttaacatcttccagtgtggtgccgttcttatagacagttatcacttacttactgtagcccattgcgtttacaagtttacgcttgaaaatgcttttcccttgaaagtaagactgggagaatgggacacccaaaataccaatgagttcttgaagcatgaagattatgaagtggaaaaaatttacattcatcctaaatatgatgatgaaaggaaaaacttgtgggacgacattgctattttgaaactgaaagctgaagtttcctttggtcctcacattgacactatctgcttaccaaataatcaagaacattttgcaggtgttcagtgtgtggttactggttggggaaagaatgcctacaaaaatggttcgtactccaatgtattaagggaagtccacgtgcctgttattactaacgataggtgtcaggagcttctgaggaaaactagattaagtgaatggtacgtcttgtacgaaaactttatctgtgctggtggagaaagtaacgccgactcttgcaagggagacggaggtggtcctttaacgtgctggaggaaagatggtacttatggactggcaggtctggtatcatggggaattaactgtggtagtcctaatgtgcctggtgtttatgtcagagtctcaaattatcttgactggattaccaagattaccggtcgtccaatttctgattactggccacgttcgtaa

SEQ ID NO: 27 - DNA, 1185 bp, Tachypleus tridentatus
  source 1..1185: mol_type = genomic DNA
atgaaagtgttgttgttggtggctttccttttgggaacgacgttggcttatccacaagacgatgacgggccagtctggggtggttcaagcaacgataatgatgatggtggtattagcagtcgcgttggcaacccccaatctggttttggtaactgtgagtgtgtaccttattacttgtgtaaggataataatattatcattgatggttctggcttactcgaccctagaaaaaaaccagtagcctccaaagaacctaaattgtctgcacgcctaggtccagaaggtccaagtgggtgtggtccttttcacgtatgctgtattgcaccagaaacatccacagtaaaaccatatactcatcaatgtggcttcagaaacgtcaatggaatcaacaagcgtattttgagtcctaatggtaaagatctatctgagtttggagagtggccttggcagggagctgtattgaaagtcgaaggcaaagttaacatcttccagtgtggtgccgttcttatagacagttatcacttacttactgtagcccattgcgtttacaagtttacgcttgaaaatgcttttcccttgaaagtaagactgggagaatgggacacccaaaataccaatgagttcttgaagcatgaagattatgaagtggaaaaaatttacattcatcctaaatatgatgatgaaaggaaaaacttgtgggacgacattgctattttgaaactgaaagctgaagtttcctttggtcctcacattgacactatctgcttaccaaataatcaagaacattttgcaggtgttcagtgtgtggttactggttggggaaagaatgcctacaaaaatggttcgtactccaatgtattaagggaagtccacgtgcctgttattactaacgataggtgtcaggagcttctcagaaaaactaggttaagtgaatggtacgtcttgtacgaaaactttatctgtgctggtggagaaagtaacgctgactcttgcaagggagatggaggtggtcctttaacgtgctggaggaaagatggtacttatggactagcaggtctggtatcatggggaattaactgtggtagtcctaatgtgcctggtgtttatgtcagagttgcaaattatcttgactggattaccaagattaccggtcgtccaatttctgattactggccacgttcgtaa

SEQ ID NO: 28 - DNA, 1242 bp, Tachypleus tridentatus
  source 1..1242: mol_type = genomic DNA
atggggatccttcccagccctgggatgcctgcgctgctctccctcgtgagccttctctccgtgctgctgatgggttgcgtagctgaaaccggtcaagacgatgacgggccagtctggggtggttcaagcaacgataatgatgatggtggtattagcagtcgcgttggcaacccccaatctggttttggtaactgtgagtgtgtaccttattacttgtgtaaggataataatattatcattgatggttctggcttactcgaccctagaaaaaaaccagtagcctccaaagaacctaaattgtctgcacgcctaggtccagaaggtccaagtgggtgtggtccttttcacgtatgctgtattgcaccagaaacatccacagtaaaaccatatactcatcaatgtggcttcagaaacgtcaatggaatcaacaagcgtattttgagtcctaatggtaaagatctatctgagtttggagagtggccttggcagggagctgtattgaaagtcgaaggcaaagttaacatcttccagtgtggtgccgttcttatagacagttatcacttacttactgtagcccattgcgtttacaagtttacgcttgaaaatgcttttcccttgaaagtaagactgggagaatgggacacccaaaataccaatgagttcttgaagcatgaagattatgaagtggaaaaaatttacattcatcctaaatatgatgatgaaaggaaaaacttgtgggacgacattgctattttgaaactgaaagctgaagtttcctttggtcctcacattgacactatctgcttaccaaataatcaagaacattttgcaggtgttcagtgtgtggttactggttggggaaagaatgcctacaaaaatggttcgtactccaatgtattaagggaagtccacgtgcctgttattactaacgataggtgtcaggagcttctcagaaaaactaggttaagtgaatggtacgtcttgtacgaaaactttatctgtgctggtggagaaagtaacgctgactcttgcaagggagatggaggtggtcctttaacgtgctggaggaaagatggtacttatggactagcaggtctggtatcatggggaattaactgtggtagtcctaatgtgcctggtgtttatgtcagagttgcaaattatcttgactggattaccaagattaccggtcgtccaatttctgattactggccacgttcgcaccaccatcaccatcactaa

SEQ ID NO: 29 - DNA, 1185 bp, Limulus polyphemus
  source 1..1185: mol_type = genomic DNA
atgaaagtgttgttgctgatgactttcctttttgaaacggcgttggcttatccacaagacgatgacggaccaatctggggtggttcaaacagcgataacgatgacgggagtattaatagtcgagttgacaacccccactccggttttggtaattgcgagtgtgtaccttattacgtgtgtaaggacgacaatatcatcactgatggttctggcgtactcgaccctaggaaaaaaccagtaccctccaaagaacccgatttgtttgcccacctgagtccagaaggccgaagagggtgtggtaactttcatgtatgttgtattgcaccaacaacatccaccgtaaaaccatatactcgtcaatgtggcttcaggaaagtcaatggcatcaacaagcgtattttgagtcctaatggtaaaaatctgtccgagtttggagagtggccttggcagggagctgtcctaaaagtcgaaggcaaagttaacatcttccagtgtggtgccgttcttatagacagttttcacttgcttactgtagcccattgcgtttacagatttacgcttgaaaatgcttttcctttgaaagtgcgactgggagaatgggatacccaaaatactaatgagttcttgaagcatgaagattatgaagtggaaaaaatttccatccactctaaatataatcatgaaaggaaaaacttgtgggacgacatcgctattttgaaactgaaagtggaagtttcctttggtcctcatattgacaccatctgtttaccaaaatatcaagaaaagtttgaaggtgttcagtgtgtggttactggttggggaaagaatgcctacaaaaatggttcgtacaccaatgtcttaagaaaagcccatgttcctgttattagtaacgataaatgtcagcagcttctgagaaaaactaggttaagtaagtggttcatcttgtatgaaaactttatctgtgctggtggagaaagtaacgccgattcttgcaagggggatggaggtggccccttagcctgctggagaaaagacggtacctatggattggcaggcctggtatcgtggggaattggctgcggtagtcctaatgtccctggtgtttatgtcagagttacaaattatcttgactggattacagaagttactggtcgaccgatctcggagtactggccacgttcttaa

SEQ ID NO: 30 - DNA, 1191 bp, Limulus polyphemus
  source 1..1191: mol_type = genomic DNA
atgaaagtgttgttgttgatgactttcctttttggaacggcgttggcttatccacaagacgatgacggaccagtctggggtggttcaaacaacgatgacgatgacgatgacgggggtattagtagtcgagttggcaacccacaatctagttttggtaactgcgagtgtgtaccttattacttgtgtaaggacaataatattatcactgatggttctggcgtactcgaccctaggaaaaaaccagtaccctccaaagaacccggtttgtctgcccgccttggtccagaaggtccaagtgggtgtggtccgtttcacgtatgttgcactgcgccaacaacatcaacagtaaaaccatatactcatcaatgtggcttcaggaacgtcaatgggatcaacaagcgtattttgagtcctaatggtaaagatctatctgagtttggagagtggccttggcagggtgctgtcctaaaagtcgaaggcaaagttaacatcttccagtgtggtgccgttcttatagacagttttcacttgcttactgtagcccactgcgtttacagatttacgcttgcaaatgcttttcctttgaaagtgcgactgggagaatgggatacccagaatactgatgagttcttgaagcatgaagattatgaagtggaaaaaatttacatccactctaaatataatcatgaaaggaaaaacttgtgggacgacatcgctattttgaaactgaaagtggaagtttcctttggtcctcatattgacaccatctgtttaccaaattaccaagaaaattttgaaggtgttcagtgtgtggttactggttggggaaagaatgcctacaaaaatggtacgtactccaatgtcttaagagaagtccatgtgcctgttattagtaacgataaatgtgagcagcttctgaaagaaactaggctaagtaagtggttcgtcttgtatgaaaactttacctgtgctggtggagaaagtaacgccgattcttgcaagggagatggaggtggccccttagcctgctggagaaaagatggtacttatgcattggcaggcctggtatcgtggggaattgactgcggtagtcctaatgtgcctggtgtttatgtcagagttgcaaaatatcttgattggattgcccaaattactggtcgtccggtcacggattactggccacggtcttaa

SEQ ID NO: 31 - DNA, 1248 bp, Limulus polyphemus
  source 1..1248: mol_type = genomic DNA
atggggatccttcccagccctgggatgcctgcgctgctctccctcgtgagccttctctccgtgctgctgatgggttgcgtagctgaaaccggtcaagacgatgacggaccagtctggggtggttcaaacaacgatgacgatgacgatgacgggggtattagtagtcgagttggcaacccacaatctagttttggtaactgcgagtgtgtaccttattacttgtgtaaggacaataatattatcactgatggttctggcgtactcgaccctaggaaaaaaccagtaccctccaaagaacccggtttgtctgcccgccttggtccagaaggtccaagtgggtgtggtccgtttcacgtatgttgcactgcgccaacaacatcaacagtaaaaccatatactcatcaatgtggcttcaggaacgtcaatgggatcaacaagcgtattttgagtcctaatggtaaagatctatctgagtttggagagtggccttggcagggtgctgtcctaaaagtcgaaggcaaagttaacatcttccagtgtggtgccgttcttatagacagttttcacttgcttactgtagcccactgcgtttacagatttacgcttgcaaatgcttttcctttgaaagtgcgactgggagaatgggatacccagaatactgatgagttcttgaagcatgaagattatgaagtggaaaaaatttacatccactctaaatataatcatgaaaggaaaaacttgtgggacgacatcgctattttgaaactgaaagtggaagtttcctttggtcctcatattgacaccatctgtttaccaaattaccaagaaaattttgaaggtgttcagtgtgtggttactggttggggaaagaatgcctacaaaaatggtacgtactccaatgtcttaagagaagtccatgtgcctgttattagtaacgataaatgtgagcagcttctgaaagaaactaggctaagtaagtggttcgtcttgtatgaaaactttacctgtgctggtggagaaagtaacgccgattcttgcaagggagatggaggtggccccttagcctgctggagaaaagatggtacttatgcattggcaggcctggtatcgtggggaattgactgcggtagtcctaatgtgcctggtgtttatgtcagagttgcaaaatatcttgattggattgcccaaattactggtcgtccggtcacggattactggccacggtctcaccaccatcaccatcactaa

SEQ ID NO: 32 - protein, 409 aa, Limulus polyphemus
MGILPSPGMPALLSLVSLLSVLLMGCVAETGQDDDGPVWGGSNNDDDDDDGGISSRVGNPQSSFGNCECVPYYLCKDNNIITDGSGVLDPRKKPVPSKEPGLSARLGPEGPSGCGPFHVCCTAPTTSTVKPYTHQCGFRNVNGINKRILSPNGKDLSEFGEWPWQGAVLKVEGKVNIFQCGAVLIDSFHLLTVAHCVYRFTLANAFPLKVRLGEWDTQNTDEFLKHEDYEVEKIYIHSKYNHERKNLWDDIAILKLKVEVSFGPHIDTICLPNYQENFEGVQCVVTGWGKNAYKNGTYSNVLREVHVPVISNDKCEQLLKETRLSKWFVLYENFTCAGGESNADSCKGDGGGPLACWRKDGTYALAGLVSWGIDCGSPNVPGVYVRVAKYLDWIAQITGRPVTDYWPRS

SEQ ID NO: 33 - protein, 381 aa, Limulus polyphemus
ETGQDDDGPVWGGSNNDDDDDDGGISSRVGNPQSSFGNCECVPYYLCKDNNIITDGSGVLDPRKKPVPSKEPGLSARLGPEGPSGCGPFHVCCTAPTTSTVKPYTHQCGFRNVNGINKRILSPNGKDLSEFGEWPWQGAVLKVEGKVNIFQCGAVLIDSFHLLTVAHCVYRFTLANAFPLKVRLGEWDTQNTDEFLKHEDYEVEKIYIHSKYNHERKNLWDDIAILKLKVEVSFGPHIDTICLPNYQENFEGVQCVVTGWGKNAYKNGTYSNVLREVHVPVISNDKCEQLLKETRLSKWFVLYENFTCAGGESNADSCKGDGGGPLACWRKDGTYALAGLVSWGIDCGSPNVPGVYVRVAKYLDWIAQITGRPVTDYWPRS

SEQ ID NO: 34 - DNA, 1230 bp, Limulus polyphemus
  source 1..1230: mol_type = genomic DNA
atgggcatcctgccatcccctggcatgccagccctgctgagcctggtgtctctgctgtccgtgctgctgatgggatgcgtggctgagaccggccaggacgatgacggccccgtgtggggcggcagcaacaatgatgacgatgacgatgacggaggaatctccagcagggtgggaaaccctcagtcttcctttggcaattgcgagtgcgtgccatactatctgtgcaaggataacaatatcatcaccgacggcagcggcgtgctggatccaagaaagaagccagtgccctccaaggagcctggcctgagcgcccgcctgggccctgagggcccatctggctgtggccccttccacgtgtgctgtacagctcctaccacatccaccgtgaagccatacacacatcagtgcggctttaggaacgtgaatggcatcaacaagcggatcctgtctcccaatggcaaggacctgtccgagttcggagagtggccttggcagggagccgtgctgaaggtggagggcaaggtgaacatcttccagtgtggcgccgtgctgatcgattcttttcacctgctgaccgtggctcattgcgtgtacaggttcacactggccaacgcttttcctctgaaggtgcggctgggcgagtgggatacccagaatacagacgagttcctgaagcacgaggactatgaggtggagaaaatctacatccacagcaagtataaccatgagcggaagaatctgtgggatgacatcgccatcctgaagctgaaggtggaggtgtctttcggcccccatatcgataccatctgtctgcctaactaccaggagaattttgagggagtgcagtgcgtggtgaccggctggggcaagaacgcttacaagaatggcacatattccaacgtgctgagggaggtgcatgtgcctgtgatcagcaatgacaagtgtgagcagctgctgaaggagacccggctgtctaagtggttcgtgctgtacgagaactttacatgcgccggcggcgagagcaatgctgattcttgtaagggcgacggaggaggaccactggcttgctggagaaaggacggcacatatgccctggctggactggtgagctggggaatcgattgcggctctcccaacgtgcctggcgtgtacgtgcgcgtggccaagtatctggactggatcgctcagatcaccggcagaccagtgacagattattggccccgctcctga

SEQ ID NO: 35 - protein, 376 aa, Tachypleus tridentatus
QDDDGPVWGGSSNDNDDGGISSRVGNPQSGFGNCECVPYYLCKDNNIIIDGSGLLDPRKKPVASKEPKLSAALGPEGPSGCGPFHVCCIAPETSTVKPYTHQCGFRNVNGINKRILSPNGKDLSEFGEWPWQGAVLKVEGKVNIFQCGAVLIDSYHLLTVAHCVYKFTLENAFPLKVRLGEWDTQNTNEFLKHEDYEVEKIYIHPKYDDERKNLWDDIAILKLKAEVSFGPHIDTICLPNNQEHFAGVQCVVTGWGKNAYKNGSYSNVLREVHVPVITNDRCQELLRKTRLSEWYVLYENFICAGGESNADSCKGDGGGPLTCWRKDGTYGLAGLVSWGINCGSPNVPGVYVRVSNYLDWITKITGRPISDYWPRS

SEQ ID NO: 36 - protein, 376 aa, Tachypleus tridentatus
QDDDGPVWGGSSNDNDDGGISSRVGNPQSGFGNCECVPYYLCKDNNIIIDGSGLLDPRKKPVASKEPKLSAELGPEGPSGCGPFHVCCIAPETSTVKPYTHQCGFRNVNGINKRILSPNGKDLSEFGEWPWQGAVLKVEGKVNIFQCGAVLIDSYHLLTVAHCVYKFTLENAFPLKVRLGEWDTQNTNEFLKHEDYEVEKIYIHPKYDDERKNLWDDIAILKLKAEVSFGPHIDTICLPNNQEHFAGVQCVVTGWGKNAYKNGSYSNVLREVHVPVITNDRCQELLRKTRLSEWYVLYENFICAGGESNADSCKGDGGGPLTCWRKDGTYGLAGLVSWGINCGSPNVPGVYVRVSNYLDWITKITGRPISDYWPRS

SEQ ID NO: 37 - protein, 376 aa, Tachypleus tridentatus
QDDDGPVWGGSSNDNDDGGISSRVGNPQSGFGNCECVPYYLCKDNNIIIDGSGLLDPRKKPVASKEPKLSAPLGPEGPSGCGPFHVCCIAPETSTVKPYTHQCGFRNVNGINKRILSPNGKDLSEFGEWPWQGAVLKVEGKVNIFQCGAVLIDSYHLLTVAHCVYKFTLENAFPLKVRLGEWDTQNTNEFLKHEDYEVEKIYIHPKYDDERKNLWDDIAILKLKAEVSFGPHIDTICLPNNQEHFAGVQCVVTGWGKNAYKNGSYSNVLREVHVPVITNDRCQELLRKTRLSEWYVLYENFICAGGESNADSCKGDGGGPLTCWRKDGTYGLAGLVSWGINCGSPNVPGVYVRVSNYLDWITKITGRPISDYWPRS

SEQ ID NO: 38 - protein, 376 aa, Tachypleus tridentatus
QDDDGPVWGGSSNDNDDGGISSRVGNPQSGFGNCECVPYYLCKDNNIIIDGSGLLDPRKKPVASKEPKLSARAGPEGPSGCGPFHVCCIAPETSTVKPYTHQCGFRNVNGINKRILSPNGKDLSEFGEWPWQGAVLKVEGKVNIFQCGAVLIDSYHLLTVAHCVYKFTLENAFPLKVRLGEWDTQNTNEFLKHEDYEVEKIYIHPKYDDERKNLWDDIAILKLKAEVSFGPHIDTICLPNNQEHFAGVQCVVTGWGKNAYKNGSYSNVLREVHVPVITNDRCQELLRKTRLSEWYVLYENFICAGGESNADSCKGDGGGPLTCWRKDGTYGLAGLVSWGINCGSPNVPGVYVRVSNYLDWITKITGRPISDYWPRS

SEQ ID NO: 39 - protein, 376 aa, Tachypleus tridentatus
QDDDGPVWGGSSNDNDDGGISSRVGNPQSGFGNCECVPYYLCKDNNIIIDGSGLLDPRKKPVASKEPPLSARLGPEGPSGCGPFHVCCIAPETSTVKPYTHQCGFRNVNGINKRILSPNGKDLSEFGEWPWQGAVLKVEGKVNIFQCGAVLIDSYHLLTVAHCVYKFTLENAFPLKVRLGEWDTQNTNEFLKHEDYEVEKIYIHPKYDDERKNLWDDIAILKLKAEVSFGPHIDTICLPNNQEHFAGVQCVVTGWGKNAYKNGSYSNVLREVHVPVITNDRCQELLRKTRLSEWYVLYENFICAGGESNADSCKGDGGGPLTCWRKDGTYGLAGLVSWGINCGSPNVPGVYVRVSNYLDWITKITGRPISDYWPRS

SEQ ID NO: 40 - protein, 376 aa, Tachypleus tridentatus
QDDDGPVWGGSSNDNDDGGISSRVGNPQSGFGNCECVPYYLCKDNNIIIDGSGLLDPRKKPVASKEPKLSARLGPEGPSGCGPFHVCCIAPETSTVKPYTHQCGFRNVNGINKRILSANGKDLSEFGEWPWQGAVLKVEGKVNIFQCGAVLIDSYHLLTVAHCVYKFTLENAFPLKVRLGEWDTQNTNEFLKHEDYEVEKIYIHPKYDDERKNLWDDIAILKLKAEVSFGPHIDTICLPNNQEHFAGVQCVVTGWGKNAYKNGSYSNVLREVHVPVITNDRCQELLRKTRLSEWYVLYENFICAGGESNADSCKGDGGGPLTCWRKDGTYGLAGLVSWGINCGSPNVPGVYVRVSNYLDWITKITGRPISDYWPRS

SEQ ID NO: 41 - protein, 376 aa, Tachypleus tridentatus
QDDDGPVWGGSSNDNDDGGISSRVGNPQSGFGNCECVPYYLCKDNNIIIDGSGLLDPRKKPVASKEPKLSARLGPEGPSGCGPFHVCCIAPETSTVKPYTHQCGFRNVNGINKRILSVNGKDLSEFGEWPWQGAVLKVEGKVNIFQCGAVLIDSYHLLTVAHCVYKFTLENAFPLKVRLGEWDTQNTNEFLKHEDYEVEKIYIHPKYDDERKNLWDDIAILKLKAEVSFGPHIDTICLPNNQEHFAGVQCVVTGWGKNAYKNGSYSNVLREVHVPVITNDRCQELLRKTRLSEWYVLYENFICAGGESNADSCKGDGGGPLTCWRKDGTYGLAGLVSWGINCGSPNVPGVYVRVSNYLDWITKITGRPISDYWPRS

SEQ ID NO: 42 - protein, 376 aa, Tachypleus tridentatus
QDDDGPVWGGSSNDNDDGGISSRVGNPQSGFGNCECVPYYLCKDNNIIIDGSGLLDPRKKPVASKEPKLSARLGPEGPSGCGPFHVCCIAPETSTVKPYTHQCGFRNVNGINKRILSGNGKDLSEFGEWPWQGAVLKVEGKVNIFQCGAVLIDSYHLLTVAHCVYKFTLENAFPLKVRLGEWDTQNTNEFLKHEDYEVEKIYIHPKYDDERKNLWDDIAILKLKAEVSFGPHIDTICLPNNQEHFAGVQCVVTGWGKNAYKNGSYSNVLREVHVPVITNDRCQELLRKTRLSEWYVLYENFICAGGESNADSCKGDGGGPLTCWRKDGTYGLAGLVSWGINCGSPNVPGVYVRVSNYLDWITKITGRPISDYWPRS

SEQ ID NO: 43 - protein, 376 aa, Tachypleus tridentatus
QDDDGPVWGGSSNDNDDGGISSRVGNPQSGFGNCECVPYYLCKDNNIIIDGSGLLDPRKKPVASKEPKLSAALGPEGPSGCGPFHVCCIAPETSTVKPYTHQCGFRNVNGINKRILSPNGKDLSEFGEWPWQGAVLKVEGKVNIFQCGAVLIDSYHLLTVAHCVYKFTLENAFPLKVRLGEWDTQNTNEFLKHEDYEVEKIYIHPKYDDERKNLWDDIAILKLKAEVSFGPHIDTICLPNNQEHFAGVQCVVTGWGKNAYKNGSYSNVLREVHVPVITNDRCQELLRKTRLSEWYVLYENFICAGGESNADSCKGDGGGPLTCWRKDGTYGLAGLVSWGINCGSPNVPGVYVRVANYLDWITKITGRPISDYWPRS

SEQ ID NO: 44 - protein, 376 aa, Tachypleus tridentatus
QDDDGPVWGGSSNDNDDGGISSRVGNPQSGFGNCECVPYYLCKDNNIIIDGSGLLDPRKKPVASKEPKLSAELGPEGPSGCGPFHVCCIAPETSTVKPYTHQCGFRNVNGINKRILSPNGKDLSEFGEWPWQGAVLKVEGKVNIFQCGAVLIDSYHLLTVAHCVYKFTLENAFPLKVRLGEWDTQNTNEFLKHEDYEVEKIYIHPKYDDERKNLWDDIAILKLKAEVSFGPHIDTICLPNNQEHFAGVQCVVTGWGKNAYKNGSYSNVLREVHVPVITNDRCQELLRKTRLSEWYVLYENFICAGGESNADSCKGDGGGPLTCWRKDGTYGLAGLVSWGINCGSPNVPGVYVRVANYLDWITKITGRPISDYWPRS

SEQ ID NO: 45 - protein, 376 aa, Tachypleus tridentatus
QDDDGPVWGGSSNDNDDGGISSRVGNPQSGFGNCECVPYYLCKDNNIIIDGSGLLDPRKKPVASKEPKLSAPLGPEGPSGCGPFHVCCIAPETSTVKPYTHQCGFRNVNGINKRILSPNGKDLSEFGEWPWQGAVLKVEGKVNIFQCGAVLIDSYHLLTVAHCVYKFTLENAFPLKVRLGEWDTQNTNEFLKHEDYEVEKIYIHPKYDDERKNLWDDIAILKLKAEVSFGPHIDTICLPNNQEHFAGVQCVVTGWGKNAYKNGSYSNVLREVHVPVITNDRCQELLRKTRLSEWYVLYENFICAGGESNADSCKGDGGGPLTCWRKDGTYGLAGLVSWGINCGSPNVPGVYVRVANYLDWITKITGRPISDYWPRS

SEQ ID NO: 46 - protein, 376 aa, Tachypleus tridentatus
QDDDGPVWGGSSNDNDDGGISSRVGNPQSGFGNCECVPYYLCKDNNIIIDGSGLLDPRKKPVASKEPKLSARAGPEGPSGCGPFHVCCIAPETSTVKPYTHQCGFRNVNGINKRILSPNGKDLSEFGEWPWQGAVLKVEGKVNIFQCGAVLIDSYHLLTVAHCVYKFTLENAFPLKVRLGEWDTQNTNEFLKHEDYEVEKIYIHPKYDDERKNLWDDIAILKLKAEVSFGPHIDTICLPNNQEHFAGVQCVVTGWGKNAYKNGSYSNVLREVHVPVITNDRCQELLRKTRLSEWYVLYENFICAGGESNADSCKGDGGGPLTCWRKDGTYGLAGLVSWGINCGSPNVPGVYVRVANYLDWITKITGRPISDYWPRS

SEQ ID NO: 47 - protein, 376 aa, Tachypleus tridentatus
QDDDGPVWGGSSNDNDDGGISSRVGNPQSGFGNCECVPYYLCKDNNIIIDGSGLLDPRKKPVASKEPPLSARLGPEGPSGCGPFHVCCIAPETSTVKPYTHQCGFRNVNGINKRILSPNGKDLSEFGEWPWQGAVLKVEGKVNIFQCGAVLIDSYHLLTVAHCVYKFTLENAFPLKVRLGEWDTQNTNEFLKHEDYEVEKIYIHPKYDDERKNLWDDIAILKLKAEVSFGPHIDTICLPNNQEHFAGVQCVVTGWGKNAYKNGSYSNVLREVHVPVITNDRCQELLRKTRLSEWYVLYENFICAGGESNADSCKGDGGGPLTCWRKDGTYGLAGLVSWGINCGSPNVPGVYVRVANYLDWITKITGRPISDYWPRS

SEQ ID NO: 48 - protein, 376 aa, Tachypleus tridentatus
QDDDGPVWGGSSNDNDDGGISSRVGNPQSGFGNCECVPYYLCKDNNIIIDGSGLLDPRKKPVASKEPKLSARLGPEGPSGCGPFHVCCIAPETSTVKPYTHQCGFRNVNGINKRILSANGKDLSEFGEWPWQGAVLKVEGKVNIFQCGAVLIDSYHLLTVAHCVYKFTLENAFPLKVRLGEWDTQNTNEFLKHEDYEVEKIYIHPKYDDERKNLWDDIAILKLKAEVSFGPHIDTICLPNNQEHFAGVQCVVTGWGKNAYKNGSYSNVLREVHVPVITNDRCQELLRKTRLSEWYVLYENFICAGGESNADSCKGDGGGPLTCWRKDGTYGLAGLVSWGINCGSPNVPGVYVRVANYLDWITKITGRPISDYWPRS

SEQ ID NO: 49 - protein, 376 aa, Tachypleus tridentatus
QDDDGPVWGGSSNDNDDGGISSRVGNPQSGFGNCECVPYYLCKDNNIIIDGSGLLDPRKKPVASKEPKLSARLGPEGPSGCGPFHVCCIAPETSTVKPYTHQCGFRNVNGINKRILSVNGKDLSEFGEWPWQGAVLKVEGKVNIFQCGAVLIDSYHLLTVAHCVYKFTLENAFPLKVRLGEWDTQNTNEFLKHEDYEVEKIYIHPKYDDERKNLWDDIAILKLKAEVSFGPHIDTICLPNNQEHFAGVQCVVTGWGKNAYKNGSYSNVLREVHVPVITNDRCQELLRKTRLSEWYVLYENFICAGGESNADSCKGDGGGPLTCWRKDGTYGLAGLVSWGINCGSPNVPGVYVRVANYLDWITKITGRPISDYWPRS

SEQ ID NO: 50 - protein, 376 aa, Tachypleus tridentatus
QDDDGPVWGGSSNDNDDGGISSRVGNPQSGFGNCECVPYYLCKDNNIIIDGSGLLDPRKKPVASKEPKLSARLGPEGPSGCGPFHVCCIAPETSTVKPYTHQCGFRNVNGINKRILSGNGKDLSEFGEWPWQGAVLKVEGKVNIFQCGAVLIDSYHLLTVAHCVYKFTLENAFPLKVRLGEWDTQNTNEFLKHEDYEVEKIYIHPKYDDERKNLWDDIAILKLKAEVSFGPHIDTICLPNNQEHFAGVQCVVTGWGKNAYKNGSYSNVLREVHVPVITNDRCQELLRKTRLSEWYVLYENFICAGGESNADSCKGDGGGPLTCWRKDGTYGLAGLVSWGINCGSPNVPGVYVRVANYLDWITKITGRPISDYWPRS

SEQ ID NO: 51 - protein, 376 aa, Limulus polyphemus
QDDDGPIWGGSNSDNDDGSINSRVDNPHSGFGNCECVPYYVCKDDNIITDGSGVLDPRKKPVPSKEPDLFAALSPEGRRGCGNFHVCCIAPTTSTVKPYTRQCGFRKVNGINKRILSPNGKNLSEFGEWPWQGAVLKVEGKVNIFQCGAVLIDSFHLLTVAHCVYRFTLENAFPLKVRLGEWDTQNTNEFLKHEDYEVEKISIHSKYNHERKNLWDDIAILKLKVEVSFGPHIDTICLPKYQEKFEGVQCVVTGWGKNAYKNGSYTNVLRKAHVPVISNDKCQQLLRKTRLSKWFILYENFICAGGESNADSCKGDGGGPLACWRKDGTYGLAGLVSWGIGCGSPNVPGVYVRVTNYLDWITEVTGRPISEYWPRS

SEQ ID NO: 52 - protein, 376 aa, Limulus polyphemus
QDDDGPIWGGSNSDNDDGSINSRVDNPHSGFGNCECVPYYVCKDDNIITDGSGVLDPRKKPVPSKEPDLFAELSPEGRRGCGNFHVCCIAPTTSTVKPYTRQCGFRKVNGINKRILSPNGKNLSEFGEWPWQGAVLKVEGKVNIFQCGAVLIDSFHLLTVAHCVYRFTLENAFPLKVRLGEWDTQNTNEFLKHEDYEVEKISIHSKYNHERKNLWDDIAILKLKVEVSFGPHIDTICLPKYQEKFEGVQCVVTGWGKNAYKNGSYTNVLRKAHVPVISNDKCQQLLRKTRLSKWFILYENFICAGGESNADSCKGDGGGPLACWRKDGTYGLAGLVSWGIGCGSPNVPGVYVRVTNYLDWITEVTGRPISEYWPRS

SEQ ID NO: 53 - protein, 376 aa, Limulus polyphemus
QDDDGPIWGGSNSDNDDGSINSRVDNPHSGFGNCECVPYYVCKDDNIITDGSGVLDPRKKPVPSKEPDLFAPLSPEGRRGCGNFHVCCIAPTTSTVKPYTRQCGFRKVNGINKRILSPNGKNLSEFGEWPWQGAVLKVEGKVNIFQCGAVLIDSFHLLTVAHCVYRFTLENAFPLKVRLGEWDTQNTNEFLKHEDYEVEKISIHSKYNHERKNLWDDIAILKLKVEVSFGPHIDTICLPKYQEKFEGVQCVVTGWGKNAYKNGSYTNVLRKAHVPVISNDKCQQLLRKTRLSKWFILYENFICAGGESNADSCKGDGGGPLACWRKDGTYGLAGLVSWGIGCGSPNVPGVYVRVTNYLDWITEVTGRPISEYWPRS

SEQ ID NO: 54 - protein, 376 aa, Limulus polyphemus
QDDDGPIWGGSNSDNDDGSINSRVDNPHSGFGNCECVPYYVCKDDNIITDGSGVLDPRKKPVPSKEPDLFAHASPEGRRGCGNFHVCCIAPTTSTVKPYTRQCGFRKVNGINKRILSPNGKNLSEFGEWPWQGAVLKVEGKVNIFQCGAVLIDSFHLLTVAHCVYRFTLENAFPLKVRLGEWDTQNTNEFLKHEDYEVEKISIHSKYNHERKNLWDDIAILKLKVEVSFGPHIDTICLPKYQEKFEGVQCVVTGWGKNAYKNGSYTNVLRKAHVPVISNDKCQQLLRKTRLSKWFILYENFICAGGESNADSCKGDGGGPLACWRKDGTYGLAGLVSWGIGCGSPNVPGVYVRVTNYLDWITEVTGRPISEYWPRS

SEQ ID NO: 55 - protein, 376 aa, Limulus polyphemus
QDDDGPIWGGSNSDNDDGSINSRVDNPHSGFGNCECVPYYVCKDDNIITDGSGVLDPRKKPVPSKEPPLFAHLSPEGRRGCGNFHVCCIAPTTSTVKPYTRQCGFRKVNGINKRILSPNGKNLSEFGEWPWQGAVLKVEGKVNIFQCGAVLIDSFHLLTVAHCVYRFTLENAFPLKVRLGEWDTQNTNEFLKHEDYEVEKISIHSKYNHERKNLWDDIAILKLKVEVSFGPHIDTICLPKYQEKFEGVQCVVTGWGKNAYKNGSYTNVLRKAHVPVISNDKCQQLLRKTRLSKWFILYENFICAGGESNADSCKGDGGGPLACWRKDGTYGLAGLVSWGIGCGSPNVPGVYVRVTNYLDWITEVTGRPISEYWPRS

SEQ ID NO: 56 - protein, 376 aa, Limulus polyphemus
QDDDGPIWGGSNSDNDDGSINSRVDNPHSGFGNCECVPYYVCKDDNIITDGSGVLDPRKKPVPSKEPDLFAHLSPEGRRGCGNFHVCCIAPTTSTVKPYTRQCGFRKVNGINKRILSANGKNLSEFGEWPWQGAVLKVEGKVNIFQCGAVLIDSFHLLTVAHCVYRFTLENAFPLKVRLGEWDTQNTNEFLKHEDYEVEKISIHSKYNHERKNLWDDIAILKLKVEVSFGPHIDTICLPKYQEKFEGVQCVVTGWGKNAYKNGSYTNVLRKAHVPVISNDKCQQLLRKTRLSKWFILYENFICAGGESNADSCKGDGGGPLACWRKDGTYGLAGLVSWGIGCGSPNVPGVYVRVTNYLDWITEVTGRPISEYWPRS

SEQ ID NO: 57 - protein, 376 aa, Limulus polyphemus
QDDDGPIWGGSNSDNDDGSINSRVDNPHSGFGNCECVPYYVCKDDNIITDGSGVLDPRKKPVPSKEPDLFAHLSPEGRRGCGNFHVCCIAPTTSTVKPYTRQCGFRKVNGINKRILSVNGKNLSEFGEWPWQGAVLKVEGKVNIFQCGAVLIDSFHLLTVAHCVYRFTLENAFPLKVRLGEWDTQNTNEFLKHEDYEVEKISIHSKYNHERKNLWDDIAILKLKVEVSFGPHIDTICLPKYQEKFEGVQCVVTGWGKNAYKNGSYTNVLRKAHVPVISNDKCQQLLRKTRLSKWFILYENFICAGGESNADSCKGDGGGPLACWRKDGTYGLAGLVSWGIGCGSPNVPGVYVRVTNYLDWITEVTGRPISEYWPRS

SEQ ID NO: 58 - protein, 376 aa, Limulus polyphemus
QDDDGPIWGGSNSDNDDGSINSRVDNPHSGFGNCECVPYYVCKDDNIITDGSGVLDPRKKPVPSKEPDLFAHLSPEGRRGCGNFHVCCIAPTTSTVKPYTRQCGFRKVNGINKRILSGNGKNLSEFGEWPWQGAVLKVEGKVNIFQCGAVLIDSFHLLTVAHCVYRFTLENAFPLKVRLGEWDTQNTNEFLKHEDYEVEKISIHSKYNHERKNLWDDIAILKLKVEVSFGPHIDTICLPKYQEKFEGVQCVVTGWGKNAYKNGSYTNVLRKAHVPVISNDKCQQLLRKTRLSKWFILYENFICAGGESNADSCKGDGGGPLACWRKDGTYGLAGLVSWGIGCGSPNVPGVYVRVTNYLDWITEVTGRPISEYWPRS

SEQ ID NO: 59 - protein, 378 aa, Limulus polyphemus
QDDDGPVWGGSNNDDDDDDGGISSRVGNPQSSFGNCECVPYYLCKDNNIITDGSGVLDPRKKPVPSKEPGLSAALGPEGPSGCGPFHVCCTAPTTSTVKPYTHQCGFRNVNGINKRILSPNGKDLSEFGEWPWQGAVLKVEGKVNIFQCGAVLIDSFHLLTVAHCVYRFTLANAFPLKVRLGEWDTQNTDEFLKHEDYEVEKIYIHSKYNHERKNLWDDIAILKLKVEVSFGPHIDTICLPNYQENFEGVQCVVTGWGKNAYKNGTYSNVLREVHVPVISNDKCEQLLKETRLSKWFVLYENFTCAGGESNADSCKGDGGGPLACWRKDGTYALAGLVSWGIDCGSPNVPGVYVRVAKYLDWIAQITGRPVTDYWPRS

SEQ ID NO: 60 - protein, 378 aa, Limulus polyphemus
QDDDGPVWGGSNNDDDDDDGGISSRVGNPQSSFGNCECVPYYLCKDNNIITDGSGVLDPRKKPVPSKEPGLSAELGPEGPSGCGPFHVCCTAPTTSTVKPYTHQCGFRNVNGINKRILSPNGKDLSEFGEWPWQGAVLKVEGKVNIFQCGAVLIDSFHLLTVAHCVYRFTLANAFPLKVRLGEWDTQNTDEFLKHEDYEVEKIYIHSKYNHERKNLWDDIAILKLKVEVSFGPHIDTICLPNYQENFEGVQCVVTGWGKNAYKNGTYSNVLREVHVPVISNDKCEQLLKETRLSKWFVLYENFTCAGGESNADSCKGDGGGPLACWRKDGTYALAGLVSWGIDCGSPNVPGVYVRVAKYLDWIAQITGRPVTDYWPRS

SEQ ID NO: 61 - protein, 378 aa, Limulus polyphemus
QDDDGPVWGGSNNDDDDDDGGISSRVGNPQSSFGNCECVPYYLCKDNNIITDGSGVLDPRKKPVPSKEPGLSAPLGPEGPSGCGPFHVCCTAPTTSTVKPYTHQCGFRNVNGINKRILSPNGKDLSEFGEWPWQGAVLKVEGKVNIFQCGAVLIDSFHLLTVAHCVYRFTLANAFPLKVRLGEWDTQNTDEFLKHEDYEVEKIYIHSKYNHERKNLWDDIAILKLKVEVSFGPHIDTICLPNYQENFEGVQCVVTGWGKNAYKNGTYSNVLREVHVPVISNDKCEQLLKETRLSKWFVLYENFTCAGGESNADSCKGDGGGPLACWRKDGTYALAGLVSWGIDCGSPNVPGVYVRVAKYLDWIAQITGRPVTDYWPRS

SEQ ID NO: 62 - protein, 378 aa, Limulus polyphemus
QDDDGPVWGGSNNDDDDDDGGISSRVGNPQSSFGNCECVPYYLCKDNNIITDGSGVLDPRKKPVPSKEPGLSARAGPEGPSGCGPFHVCCTAPTTSTVKPYTHQCGFRNVNGINKRILSPNGKDLSEFGEWPWQGAVLKVEGKVNIFQCGAVLIDSFHLLTVAHCVYRFTLANAFPLKVRLGEWDTQNTDEFLKHEDYEVEKIYIHSKYNHERKNLWDDIAILKLKVEVSFGPHIDTICLPNYQENFEGVQCVVTGWGKNAYKNGTYSNVLREVHVPVISNDKCEQLLKETRLSKWFVLYENFTCAGGESNADSCKGDGGGPLACWRKDGTYALAGLVSWGIDCGSPNVPGVYVRVAKYLDWIAQITGRPVTDYWPRS

SEQ ID NO: 63 - protein, 378 aa, Limulus polyphemus
QDDDGPVWGGSNNDDDDDDGGISSRVGNPQSSFGNCECVPYYLCKDNNIITDGSGVLDPRKKPVPSKEPPLSARLGPEGPSGCGPFHVCCTAPTTSTVKPYTHQCGFRNVNGINKRILSPNGKDLSEFGEWPWQGAVLKVEGKVNIFQCGAVLIDSFHLLTVAHCVYRFTLANAFPLKVRLGEWDTQNTDEFLKHEDYEVEKIYIHSKYNHERKNLWDDIAILKLKVEVSFGPHIDTICLPNYQENFEGVQCVVTGWGKNAYKNGTYSNVLREVHVPVISNDKCEQLLKETRLSKWFVLYENFTCAGGESNADSCKGDGGGPLACWRKDGTYALAGLVSWGIDCGSPNVPGVYVRVAKYLDWIAQITGRPVTDYWPRS

SEQ ID NO: 64 - protein, 378 aa, Limulus polyphemus
QDDDGPVWGGSNNDDDDDDGGISSRVGNPQSSFGNCECVPYYLCKDNNIITDGSGVLDPRKKPVPSKEPGLSARLGPEGPSGCGPFHVCCTAPTTSTVKPYTHQCGFRNVNGINKRILSANGKDLSEFGEWPWQGAVLKVEGKVNIFQCGAVLIDSFHLLTVAHCVYRFTLANAFPLKVRLGEWDTQNTDEFLKHEDYEVEKIYIHSKYNHERKNLWDDIAILKLKVEVSFGPHIDTICLPNYQENFEGVQCVVTGWGKNAYKNGTYSNVLREVHVPVISNDKCEQLLKETRLSKWFVLYENFTCAGGESNADSCKGDGGGPLACWRKDGTYALAGLVSWGIDCGSPNVPGVYVRVAKYLDWIAQITGRPVTDYWPRS

SEQ ID NO: 65 - protein, 378 aa, Limulus polyphemus
QDDDGPVWGGSNNDDDDDDGGISSRVGNPQSSFGNCECVPYYLCKDNNIITDGSGVLDPRKKPVPSKEPGLSARLGPEGPSGCGPFHVCCTAPTTSTVKPYTHQCGFRNVNGINKRILSVNGKDLSEFGEWPWQGAVLKVEGKVNIFQCGAVLIDSFHLLTVAHCVYRFTLANAFPLKVRLGEWDTQNTDEFLKHEDYEVEKIYIHSKYNHERKNLWDDIAILKLKVEVSFGPHIDTICLPNYQENFEGVQCVVTGWGKNAYKNGTYSNVLREVHVPVISNDKCEQLLKETRLSKWFVLYENFTCAGGESNADSCKGDGGGPLACWRKDGTYALAGLVSWGIDCGSPNVPGVYVRVAKYLDWIAQITGRPVTDYWPRS

SEQ ID NO: 66 - protein, 378 aa, Limulus polyphemus
QDDDGPVWGGSNNDDDDDDGGISSRVGNPQSSFGNCECVPYYLCKDNNIITDGSGVLDPRKKPVPSKEPGLSARLGPEGPSGCGPFHVCCTAPTTSTVKPYTHQCGFRNVNGINKRILSGNGKDLSEFGEWPWQGAVLKVEGKVNIFQCGAVLIDSFHLLTVAHCVYRFTLANAFPLKVRLGEWDTQNTDEFLKHEDYEVEKIYIHSKYNHERKNLWDDIAILKLKVEVSFGPHIDTICLPNYQENFEGVQCVVTGWGKNAYKNGTYSNVLREVHVPVISNDKCEQLLKETRLSKWFVLYENFTCAGGESNADSCKGDGGGPLACWRKDGTYALAGLVSWGIDCGSPNVPGVYVRVAKYLDWIAQITGRPVTDYWPRS

SEQ ID NO: 67 - protein, 394 aa, Carcinoscorpius rotundicauda
MKVLLVAFLLGTTLAYPQDDDGPVWGGSSNDDDDDGGISSRIGNPQSGFGNCECVPYYLCKDNNIIIDGSGLLDPRKKPVASKEPELSARLGPEGPSGCGPFHVCCIAPETSTVKPYTHQCGFRNVNGINKRILSPNGKDLSEFGEWPWQGAVLKIEGKVNIFQCGAVLIDSYHLLTVAHCVYKFTLENAFPLKVRLGEWDTQNTNEFLKHEDYEVEKIYIHDKYDHERKNLWDDIAILKLKTEVSFGPHIDTICLPNNEEHFAGVQCVVTGWGKNAYKNGSYSNVLREVHMPVITNDRCQELLRETRLSKWFVLYKNFVCAGGESNTDSCKGDGGGPLACWRKDGTYGLAGLVSWGIDCGSPNVPGVYVRVANYLDWITKITGRPISDYWPRS

SEQ ID NO: 68 - protein, 377 aa, Carcinoscorpius rotundicauda
QDDDGPVWGGSSNDDDDDGGISSRIGNPQSGFGNCECVPYYLCKDNNIIIDGSGLLDPRKKPVASKEPELSARLGPEGPSGCGPFHVCCIAPETSTVKPYTHQCGFRNVNGINKRILSPNGKDLSEFGEWPWQGAVLKIEGKVNIFQCGAVLIDSYHLLTVAHCVYKFTLENAFPLKVRLGEWDTQNTNEFLKHEDYEVEKIYIHDKYDHERKNLWDDIAILKLKTEVSFGPHIDTICLPNNEEHFAGVQCVVTGWGKNAYKNGSYSNVLREVHMPVITNDRCQELLRETRLSKWFVLYKNFVCAGGESNTDSCKGDGGGPLACWRKDGTYGLAGLVSWGIDCGSPNVPGVYVRVANYLDWITKITGRPISDYWPRS

SEQ ID NO: 69 - protein, 393 aa, Tachypleus gigas
MKVLLLVAFLLGTTLAYPQDDDGPVWGSNDNDDDGGISSRVGNPQSGFGNCVCVPYYLCKDNNIIIDGSGLLDPRKKPIATKEPELSARLGPEGPSGCGPFHVCCIAPETSTVKPYTHQCGFRNVNGINKRILSPNGKDLSEFGEWPWQGAVLKVEGKVNIFQCGAVLIDSYHLLTVAHCVYKFTLENAFPLKVRLGEWDTQNTNEFLKHEDYEVEKIYVHPKYDHERKNLWDDIAVLKLKAEVSFGPHIDTICLPNNQEHFAGVQCVVTGWGKNAYKNGSYSNVLREVHMPVITNERCQELLKKTRLSEWFVLYENFICAGGESNTDSCKGDGGGPLACWRKDGTYGLAGLVSWGIDCGSPNVPGVYVRVSNYLDWITKVTGRPISDYWPRS

SEQ ID NO: 70 - protein, 375 aa, Tachypleus gigas
QDDDGPVWGSNDNDDDGGISSRVGNPQSGFGNCVCVPYYLCKDNNIIIDGSGLLDPRKKPIATKEPELSARLGPEGPSGCGPFHVCCIAPETSTVKPYTHQCGFRNVNGINKRILSPNGKDLSEFGEWPWQGAVLKVEGKVNIFQCGAVLIDSYHLLTVAHCVYKFTLENAFPLKVRLGEWDTQNTNEFLKHEDYEVEKIYVHPKYDHERKNLWDDIAVLKLKAEVSFGPHIDTICLPNNQEHFAGVQCVVTGWGKNAYKNGSYSNVLREVHMPVITNERCQELLKKTRLSEWFVLYENFICAGGESNTDSCKGDGGGPLACWRKDGTYGLAGLVSWGIDCGSPNVPGVYVRVSNYLDWITKVTGRPISDYWPRS

SEQ ID NO: 71 - DNA, 1185 bp, Carcinoscorpius rotundicauda
  source 1..1185: mol_type = genomic DNA
atgaaagtgttgttggtggctttccttttgggaacgacgttggcttatccacaagacgatgacgggccagtctggggtggttcaagcaacgatgatgatgatgatggtggtattagcagtcgaattggcaacccccaatctggttttggtaactgcgagtgtgtaccttattacttgtgtaaggataacaatattatcattgatggttctggcttactcgacccaagaaaaaaaccagttgcctccaaagaacctgaattgtctgcacgcctaggtccagaaggtccaagtgggtgtggtccttttcacgtatgctgtattgcaccagaaacgtccacggtaaaaccatatactcatcaatgtggcttcagaaacgtcaatggaatcaacaagcgtattttgagtcctaatggtaaagatctatctgagtttggagagtggccttggcagggagctgtattgaaaatcgaaggcaaagttaacatcttccagtgtggtgccgttctcatagacagttatcacttacttactgtagcccattgcgtttacaagtttacgcttgaaaatgcttttcccttgaaagtaagactgggagaatgggatacccaaaataccaatgagttcttgaagcatgaagattatgaagtggaaaaaatttacattcatgataaatatgatcatgaaaggaaaaacttgtgggacgacattgctattttgaaactgaaaactgaagtgtcctttggtcctcacattgacactatctgcttaccaaataatgaagaacattttgcgggtgttcagtgtgtggttactggttggggaaagaatgcctacaaaaatggttcgtactccaatgtattaagggaagtccacatgcctgttattactaacgataggtgtcaggagcttctcagagaaactagattaagtaaatggttcgtcttgtacaaaaactttgtctgtgctggtggagaaagtaacaccgattcttgcaagggagatggaggtggtcctttagcctgctggaggaaagatggtacttatggactagcaggtctggtatcgtggggaattgactgtggtagtcctaatgtgcctggtgtttatgtcagagttgcaaattatcttgactggattaccaagattaccggtcgtccaatttctgattactggccacgttcgtaa

SEQ ID NO: 72 - DNA, 1182 bp, Tachypleus gigas
  source 1..1182: mol_type = genomic DNA
atgaaagtgttgttgttggtggctttccttttgggaacgacgttggcttatccacaagacgacgacgggccagtctggggtagcaacgataatgatgatgatggtggtattagcagtcgcgttggcaacccccaatctggttttggtaactgcgtgtgtgtaccttattacttgtgtaaggataataatataatcattgatggttctggcttactcgaccctagaaaaaaaccaatagccaccaaagaacctgaattgtctgcacgcctaggtccagaaggtccaagtgggtgtggtccttttcacgtatgctgtattgcaccagaaacatccacagtgaaaccatatactcatcaatgtggcttcagaaacgtcaatggaatcaacaagcgtattttgagtcctaatggtaaagatctatctgagtttggagagtggccttggcagggagctgtattgaaagtcgaaggcaaagttaacatcttccagtgtggtgccgttcttatagacagttatcacttacttactgtagcccattgcgtttataagtttacgcttgaaaatgcttttcccttgaaagtaagactgggagaatgggatacccaaaataccaacgagttcttgaagcatgaagattatgaagtggaaaaaatttacgttcatcctaaatatgatcatgaaaggaaaaacttgtgggacgacattgctgttttgaaactgaaagctgaagtttcctttggtcctcacattgacaccatctgcttaccaaataatcaagaacattttgcaggtgttcagtgtgtggttactggttggggaaagaatgcctacaaaaatggttcgtactccaatgtattacgggaagtccacatgcctgttattaccaacgaaaggtgtcaggagcttctgaaaaaaactagattaagtgaatggttcgtcttgtacgaaaactttatctgtgctggtggagaaagtaacaccgattcttgcaagggagatggaggtggtcctttagcctgctggaggaaagatggtacttatggactggcaggtctggtatcgtgggggattgactgtggtagtcctaatgtacctggtgtttatgtcagagtttcaaattatcttgattggattaccaaggttactggtcgtccaatttctgattactggccacgttcgtaa